European Patent Application EP 4 656 247 A2, published December 3, 2025. Title: ANTI-CHEMOKIN LIKE RECEPTOR 1 ANTIBODIES AND THEIR THERAPEUTIC. Applicant: OSE IMMUNOTHERAPEUTICS. Application US 18/658,406, filed May 8, 2024. The sequence listing filed with the application follows.

SEQUENCE LISTING (152 sequences)

SEQ ID NO: 1 - protein, 373 aa, synthetic construct
  REGION 1..373: note = Synthetic sequence
MRMEDEDYNTSISYGDEYPDYLDSIVVLEDLSPLEARVTRIFLVVVYSIVCFLGILGNGLVIIIATFKMKKTVNMVWFLNLAVADFLFNVFLPIHITYAAMDYHWVFGTAMCKISNFLLIHNMFTSVFLLTIISSDRCISVLLPVWSQNHRSVRLAYMACMVIWVLAFFLSSPSLVFRDTANLHGKISCFNNFSLSTPGSSSWPTHSQMDPVGYSRHMVVTVTRFLCGFLVPVLIITACYLTIVCKLQRNRLAKTKKPFKIIVTIIITFFLCWCPYHTLNLLELHHTAMPGSVFSLGLPLATALAIANSCMNPILYVFMGQDFKKFKVALFSRLVNALSEDTGHSSYPSHRSFTKMSSMNERTSMNERETGML

SEQ ID NO: 2 - protein, 18 aa, synthetic construct
  REGION 1..18: note = Synthetic sequence
ELHHTAMPGSVFSLGLPL

SEQ ID NO: 3 - protein, 8 aa, synthetic construct
  REGION 1..8: note = Synthetic sequence
GFTFSSYG

SEQ ID NO: 4 - protein, 10 aa, synthetic construct
  REGION 1..10: note = Synthetic sequence
GFTFSSYGMS

SEQ ID NO: 5 - protein, 8 aa, synthetic construct
  REGION 1..8: note = Synthetic sequence
INRYGGST

SEQ ID NO: 6 - protein, 17 aa, synthetic construct
  REGION 1..17: note = Synthetic sequence
TINRYGGSTYYPDSVKG

SEQ ID NO: 7 - protein, 12 aa, synthetic construct
  REGION 1..12: note = Synthetic sequence
PRLIYYGNEGDS

SEQ ID NO: 8 - protein, 10 aa, synthetic construct
  REGION 1..10: note = Synthetic sequence
  SITE 2: note = misc_feature - S is selected among L or I
LXYYGNEGDS

SEQ ID NO: 9 - protein, 119 aa, synthetic construct
  REGION 1..119: note = Synthetic sequence
EVQLVASGGGLVQPGGSLKLSCAASGFTFSSYGMSWVRQTPDRRLELVATINRYGGSTYYPDSVKGRFTISRDNAKNTLYLQMSSLKSEDTAMYYCPRLIYYGNEGDSWGQGTTLTVSS

SEQ ID NO: 10 - protein, 140 aa, synthetic construct
  REGION 1..140: note = Synthetic sequence
METDTLLLWVLLLWVPGSTGDEVQLVASGGGLVQPGGSLKLSCAASGFTFSSYGMSWVRQTPDRRLELVATINRYGGSTYYPDSVKGRFTISRDNAKNTLYLQMSSLKSEDTAMYYCPRLIYYGNEGDSWGQGTTLTVSS

SEQ ID NO: 11 - protein, 5 aa, synthetic construct
  REGION 1..5: note = Synthetic sequence
SSVSF

SEQ ID NO: 12 - protein, 10 aa, synthetic construct
  REGION 1..10: note = Synthetic sequence
SASSSVSFMH

SEQ ID NO: 13 - skipped

SEQ ID NO: 14 - protein, 7 aa, synthetic construct
  REGION 1..7: note = Synthetic sequence
DTTKLTS

SEQ ID NO: 15 - protein, 10 aa, synthetic construct
  REGION 1..10: note = Synthetic sequence
QQWNSKPPLT

SEQ ID NO: 16 - protein, 108 aa, synthetic construct
  REGION 1..108: note = Synthetic sequence
QIVLTQSPAIMSASPGEKVTMTCSASSSVSFMHWYQQKSGTSPKRWIYDTTKLTSGVPARFSGSGSGTFYSLTISSMEAEDAATYYCQQWNSKPPLTFGPGTKLELKR

SEQ ID NO: 17 - protein, 129 aa, synthetic construct
  REGION 1..129: note = Synthetic sequence
METDTLLLWVLLLWVPGSTGDQIVLTQSPAIMSASPGEKVTMTCSASSSVSFMHWYQQKSGTSPKRWIYDTTKLTSGVPARFSGSGSGTFYSLTISSMEAEDAATYYCQQWNSKPPLTFGPGTKLELKR

SEQ ID NO: 18 - protein, 33 aa, synthetic construct
  REGION 1..33: note = Synthetic sequence
PYHTLNLLELHHTAMPGSVFSLGLPLATALAIA

SEQ ID NO: 19 - protein, 26 aa, synthetic construct
  REGION 1..26: note = Synthetic sequence
  VARIANT 1: note = Xaa is selected among E or Q
  VARIANT 6: note = Xaa is selected among A, E or Q
  VARIANT 9: note = Xaa is selected among G, A or S
  VARIANT 11: note = Xaa is selected among L or E
  VARIANT 12: note = Xaa is selected among V or L
  VARIANT 13: note = Xaa is selected among Q or K
  VARIANT 14: note = Xaa is selected among P or K
  VARIANT 17: note = Xaa is selected among G or A
  VARIANT 19: note = Xaa is selected among L or V
  VARIANT 20: note = Xaa is selected among K, R or V
  VARIANT 21: note = Xaa is selected among L or V
  VARIANT 24: note = Xaa is selected among A or K
XVQLVXSGXGXXXXPGXSXXXSCXAS

SEQ ID NO: 20 - protein, 119 aa, synthetic construct
  REGION 1..119: note = Synthetic sequence
EVQLVESGGGLVQPGGSLRLSCAASGFTFSSYGMSWVRQAPGKGLELVATINRYGGSTYYPDSVKGRFTISRDNSKNTLYLQMNSLRAEDTAVYYCPRLIYYGNEGDSWGQGTLVTVSS

SEQ ID NO: 21 - protein, 119 aa, synthetic construct
  REGION 1..119: note = Synthetic sequence
EVQLVESGGGLVQPGGSLRLSCAASGFTFSSYGMSWVRQAPGKGLELVATINRYGGSTYYAASVKGRFTISRDNSKNTLYLQMNSLRAEDTAVYYCPKLIYYGNEGDSWGQGTLVTVSS

SEQ ID NO: 22 - protein, 119 aa, synthetic construct
  REGION 1..119: note = Synthetic sequence
EVQLVESGGGLVQPGGSLRLSCAASGFTFSSYAMSWVRQAPGKGLELVATINRYGGSTYYAASVKGRFTISRDNSKNTLYLQMNSLRAEDTAVYYCPKLIYYGNEGDSWGQGTLVTVSS

SEQ ID NO: 23 - protein, 119 aa, synthetic construct
  REGION 1..119: note = Synthetic sequence
EVQLVESGGGLVQPGGSLRLSCAASGFTFSSYAMSWVRQAPGKGLELVSTISRSGGSTYYAASVKGRFTISRDNSKNTLYLQMNSLRAEDTAVYYCPKLIYYGNEGDSWGQGTLVTVSS

SEQ ID NO: 24 - protein, 119 aa, synthetic construct
  REGION 1..119: note = Synthetic sequence
EVQLVESGGGLVQPGGSLRLSCAASGFTFSSYAMSWVRQAPGKGLELVSTISGSGGSTYYAASVKGRFTISRDNSKNTLYLQMNSLRAEDTAVYYCAKLIYYGNEGDSWGQGTLVTVSS

SEQ ID NO: 25 - protein, 119 aa, synthetic construct
  REGION 1..119: note = Synthetic sequence
EVQLVESGGGLVQPGGSLRLSCAASGFTFSSYAMSWVRQAPGKGLEWVSTISGSGGSTYYAASVKGRFTISRDNSKNTLYLQMNSLRAEDTAVYYCAKLIYYGNEGDSWGQGTLVTVSS

SEQ ID NO: 26 - protein, 119 aa, synthetic construct
  REGION 1..119: note = Synthetic sequence
EVQLVESGGGLVQPGGSLRLSCAASGFTFSSYAMSWVRQAPGKGLEWVSTISGSGGSTYYAASVKGRFTISRDNSKNTLYLQMNSLRAEDTAVYYCAKLIYYGNEGESWGQGTLVTVSS

SEQ ID NO: 27 - protein, 119 aa, synthetic construct
  REGION 1..119: note = Synthetic sequence
EVQLVESGGGLVQPGGSLRLSCAASGFTFSSYAMSWVRQAPGKGLEWVSTISGSGGSTYYAASVKGRFTISRDNSKNTLYLQMNSLRAEDTAVYYCAKLIYYGNEGDTWGQGTLVTVSS

SEQ ID NO: 28 - protein, 119 aa, synthetic construct
  REGION 1..119: note = Synthetic sequence
QVQLVQSGAEVKKPGASVKVSCKASGFTFSSYGMSWVRQAPGQGLELVATINRYGGSTYYPDSFKGRVTITRDNSTSTLYMELSSLRSEDTAVYYCPRLIYYGNEGDSWGQGTLVTVSS

SEQ ID NO: 29 - protein, 119 aa, synthetic construct
  REGION 1..119: note = Synthetic sequence
QVQLVQSGAEVKKPGASVKVSCKASGFTFSSYGMSWVRQAPGQGLELVGTINRYGGSTYYAQKFQGRVTITRDNSTSTLYMELSSLRSEDTAVYYCPRLIYYGNEGDSWGQGTLVTVSS

SEQ ID NO: 30 - protein, 119 aa, synthetic construct
  REGION 1..119: note = Synthetic sequence
QVQLVQSGAEVKKPGASVKVSCKASGYTFTSYGMSWVRQAPGQGLELMGIINRNGGSTYYAQKFQGRVTITRDTSTSTVYMELSSLRSEDTAVYYCPRLIYYGNEGDSWGQGTLVTVSS

SEQ ID NO: 31 - protein, 119 aa, synthetic construct
  REGION 1..119: note = Synthetic sequence
QVQLVQSGAEVKKPGASVKVSCKASGYTFTSYGMSWVRQAPGQGLELMGIINPNGGSTYYAQKFQGRVTITRDTSTSTVYMELSSLRSEDTAVYYCARLIYYGNEGDSWGQGTLVTVSS

SEQ ID NO: 32 - protein, 119 aa, synthetic construct
  REGION 1..119: note = Synthetic sequence
QVQLVQSGAEVKKPGASVKVSCKASGYTFTSYGMSWVRQAPGQGLEWMGIINPNGGSTYYAQKFQGRVTITRDTSTSTVYMELSSLRSEDTAVYYCARLIYYGNEGDSWGQGTLVTVSS

SEQ ID NO: 33 - protein, 119 aa, synthetic construct
  REGION 1..119: note = Synthetic sequence
QVQLVQSGAEVKKPGASVKVSCKASGYTFTSYYMHWVRQAPGQGLEWMGIINPNGGSTSYAQKFQGRVTMTRDTSTSTVYMELSSLRSEDTAVYYCARLIYYGNEGDSWGQGTLVTVSS

SEQ ID NO: 34 - protein, 119 aa, synthetic construct
  REGION 1..119: note = Synthetic sequence
QVQLVQSGAEVKKPGASVKVSCKASGYTFTSYYMHWVRQAPGQGLEWMGIINPNGGSTSYAQKFQGRVTMTRDTSTSTVYMELSSLRSEDTAVYYCARLIYYGNEGESWGQGTLVTVSS

SEQ ID NO: 35 - protein, 119 aa, synthetic construct
  REGION 1..119: note = Synthetic sequence
QVQLVQSGAEVKKPGASVKVSCKASGYTFTSYYMHWVRQAPGQGLEWMGIINPNGGSTSYAQKFQGRVTMTRDTSTSTVYMELSSLRSEDTAVYYCARLIYYGNEGDTWGQGTLVTVSS

SEQ ID NO: 36 - protein, 119 aa, synthetic construct
  REGION 1..119: note = Synthetic sequence
QVQLVQSGSELKKPGASVKVSCKASGFTFSSYGMSWVRQAPGQGLELVATINRYGGSTYYPDSFKGRFVISRDNSVSTLYLQISSLKAEDTAVYYCPRLIYYGNEGDSWGQGTLVTVSS

SEQ ID NO: 37 - protein, 119 aa, synthetic construct
  REGION 1..119: note = Synthetic sequence
QVQLVQSGSELKKPGASVKVSCKASGFTFSSYGMSWVRQAPGQGLELVGTINRYGGSPYYAQGFTGRFVISRDNSVSTLYLQISSLKAEDTAVYYCPRLIYYGNEGDSWGQGTLVTVSS

SEQ ID NO: 38 - protein, 119 aa, synthetic construct
  REGION 1..119: note = Synthetic sequence
QVQLVQSGSELKKPGASVKVSCKASGYTFTSYAMSWVRQAPGQGLELVGTINRYGGNPYYAQGFTGRFVISRDNSVSTLYLQISSLKAEDTAVYYCPRLIYYGNEGDSWGQGTLVTVSS

SEQ ID NO: 39 - protein, 119 aa, synthetic construct
  REGION 1..119: note = Synthetic sequence
QVQLVQSGSELKKPGASVKVSCKASGYTFTSYAMNWVRQAPGQGLELMGTINRYGGNPYYAQGFTGRFVISRDTSVSTAYLQISSLKAEDTAVYYCPRLIYYGNEGDSWGQGTLVTVSS

SEQ ID NO: 40 - protein, 119 aa, synthetic construct
  REGION 1..119: note = Synthetic sequence
QVQLVQSGSELKKPGASVKVSCKASGYTFTSYAMNWVRQAPGQGLELMGTINTYTGNPYYAQGFTGRFVISRDTSVSTAYLQISSLKAEDTAVYYCARLIYYGNEGDSWGQGTLVTVSS

SEQ ID NO: 41 - protein, 119 aa, synthetic construct
  REGION 1..119: note = Synthetic sequence
QVQLVQSGSELKKPGASVKVSCKASGYTFTSYAMNWVRQAPGQGLEWMGWINTYTGNPTYAQGFTGRFVISLDTSVSTAYLQISSLKAEDTAVYYCARLIYYGNEGDSWGQGTLVTVSS

SEQ ID NO: 42 - protein, 119 aa, synthetic construct
  REGION 1..119: note = Synthetic sequence
QVQLVQSGSELKKPGASVKVSCKASGYTFTSYAMNWVRQAPGQGLEWMGWINTYTGNPTYAQGFTGRFVISLDTSVSTAYLQISSLKAEDTAVYYCARLIYYGNEGETWGQGTLVTVSS

SEQ ID NO: 43 - protein, 107 aa, synthetic construct
  REGION 1..107: note = Synthetic sequence
AIQLTQSPSSLSASVGDRVTITCSASSSVSFMHWYQQKPGKAPKRWIYDTTKLTSGVPSRFSGSGSGTDYTLTISSLQPEDFATYYCQQWNSKPPLTFGGGTKVEIK

SEQ ID NO: 44 - protein, 107 aa, synthetic construct
  REGION 1..107: note = Synthetic sequence
AIQLTQSPSSLSASVGDRVTITCRASQSVSFMHWYQQKPGKAPKRWIYDATKLTSGVPSRFSGSGSGTDYTLTISSLQPEDFATYYCQQWNSKPPLTFGGGTKVEIK

SEQ ID NO: 45 - protein, 107 aa, synthetic construct
  REGION 1..107: note = Synthetic sequence
AIQLTQSPSSLSASVGDRVTITCRASQSVSFLHWYQQKPGKAPKRWIYDATKLTSGVPSRFSGSGSGTDFTLTISSLQPEDFATYYCQQWNSKPPLTFGGGTKVEIK

SEQ ID NO: 46 - protein, 107 aa, synthetic construct
  REGION 1..107: note = Synthetic sequence
AIQLTQSPSSLSASVGDRVTITCRASQSVSFLHWYQQKPGKAPKRWIYDATKLTSGVPSRFSGSGSGTDFTLTISSLQPEDFATYYCQQWQSKPPLTFGGGTKVEIK

SEQ ID NO: 47 - protein, 107 aa, synthetic construct
  REGION 1..107: note = Synthetic sequence
AIQLTQSPSSLSASVGDRVTITCRASQSVSFLHWYQQKPGKAPKRWIYDASKLTSGVPSRFSGSGSGTDFTLTISSLQPEDFATYYCQQWQSKPPLTFGGGTKVEIK

SEQ ID NO: 48 - protein, 107 aa, synthetic construct
  REGION 1..107: note = Synthetic sequence
AIQLTQSPSSLSASVGDRVTITCRASQGISFLAWYQQKPGKAPKRLIYDASKLESGVPSRFSGSGSGTDFTLTISSLQPEDFATYYCQQWQSKPPLTFGGGTKVEIK

SEQ ID NO: 49 - protein, 107 aa, synthetic construct
  REGION 1..107: note = Synthetic sequence
AIQLTQSPSSLSASVGDRVTITCRASQGISSLAWYQQKPGKAPKRLIYDASSLESGVPSRFSGSGSGTDFTLTISSLQPEDFATYYCQQFQSYPPLTFGGGTKVEIK

SEQ ID NO: 50 - protein, 107 aa, synthetic construct
  REGION 1..107: note = Synthetic sequence
EIVLTQSPDFQSVTPKEKVTITCSASSSVSFMHWYQQKPDQSPKRWIYDTTKLTSGVPSRFSGSGSGTDYTLTINSLEAEDAATYYCQQWNSKPPLTFGGGTKVEIK

SEQ ID NO: 51 - protein, 107 aa, synthetic construct
  REGION 1..107: note = Synthetic sequence
EIVLTQSPDFQSVTPKEKVTITCRASQSVSFMHWYQQKPDQSPKRWIYDATKSTSGVPSRFSGSGSGTDYTLTINSLEAEDAATYYCQQWNSKPPLTFGGGTKVEIK

SEQ ID NO: 52 - protein, 107 aa, synthetic construct
  REGION 1..107: note = Synthetic sequence
EIVLTQSPDFQSVTPKEKVTITCRASQSVSFLHWYQQKPDQSPKRWIYDATKSTSGVPSRFSGSGSGTDFTLTINSLEAEDAATYYCQQWNSKPPLTFGGGTKVEIK

SEQ ID NO: 53 - protein, 107 aa, synthetic construct
  REGION 1..107: note = Synthetic sequence
EIVLTQSPDFQSVTPKEKVTITCRASQSVSFLHWYQQKPDQSPKRWIYDATKSTSGVPSRFSGSGSGTDFTLTINSLEAEDAATYYCQQWQSKPPLTFGGGTKVEIK

SEQ ID NO: 54 - protein, 107 aa, synthetic construct
  REGION 1..107: note = Synthetic sequence
EIVLTQSPDFQSVTPKEKVTITCRASQSISFLHWYQQKPDQSPKRLIYDASKSTSGVPSRFSGSGSGTDFTLTINSLEAEDAATYYCQQWQSKPPLTFGGGTKVEIK

SEQ ID NO: 55 - protein, 107 aa, synthetic construct
  REGION 1..107: note = Synthetic sequence
EIVLTQSPDFQSVTPKEKVTITCRASQSISSLHWYQQKPDQSPKLLIYYASQSFSGVPSRFSGSGSGTDFTLTINSLEAEDAATYYCHQSQSLPPLTFGGGTKVEIK

SEQ ID NO: 56 - protein, 107 aa, synthetic construct
  REGION 1..107: note = Synthetic sequence
EIVLTQSPATLSLSPGERATLSCSASSSVSFMHWYQQKPGQAPRRWIYDTTKLTSGIPARFSGSGSGTDYTLTISSLEPEDFAVYYCQQWNSKPPLTFGGGTKVEIK

SEQ ID NO: 57 - protein, 107 aa, synthetic construct
  REGION 1..107: note = Synthetic sequence
EIVLTQSPATLSLSPGERATLSCRASQSVSFMHWYQQKPGQAPRRWIYDATKLTTGIPARFSGSGSGTDYTLTISSLEPEDFAVYYCQQWNSKPPLTFGGGTKVEIK

SEQ ID NO: 58 - protein, 107 aa, synthetic construct
  REGION 1..107: note = Synthetic sequence
EIVLTQSPATLSLSPGERATLSCRASQSVSFLHWYQQKPGQAPRRWIYDATKRTTGIPARFSGSGSGTDFTLTISSLEPEDFAVYYCQQWNSKPPLTFGGGTKVEIK

SEQ ID NO: 59 - protein, 107 aa, synthetic construct
  REGION 1..107: note = Synthetic sequence
EIVLTQSPATLSLSPGERATLSCRASQSVSFLHWYQQKPGQAPRRWIYDATKRTTGIPARFSGSGSGTDFTLTISSLEPEDFAVYYCQQWQSKPPLTFGGGTKVEIK

SEQ ID NO: 60 - protein, 107 aa, synthetic construct
  REGION 1..107: note = Synthetic sequence
EIVLTQSPATLSLSPGERATLSCRASQSVSFLAWYQQKPGQAPRRLIYDASKRTTGIPARFSGSGSGTDFTLTISSLEPEDFAVYYCQQWQSKPPLTFGGGTKVEIK

SEQ ID NO: 61 - protein, 107 aa, synthetic construct
  REGION 1..107: note = Synthetic sequence
EIVLTQSPATLSLSPGERATLSCRASQSVSYLAWYQQKPGQAPRLLIYDASNRATGIPARFSGSGSGTDFTLTISSLEPEDFAVYYCHQRQNWPPLTFGGGTKVEIK

SEQ ID NO: 62 - protein, 10 aa, synthetic construct
  REGION 1..10: note = Synthetic sequence
GFTFSSYAMS

SEQ ID NO: 63 - protein, 10 aa, synthetic construct
  REGION 1..10: note = Synthetic sequence
GYTFTSYGMS

SEQ ID NO: 64 - protein, 10 aa, synthetic construct
  REGION 1..10: note = Synthetic sequence
GYTFTSYAMS

SEQ ID NO: 65 - protein, 10 aa, synthetic construct
  REGION 1..10: note = Synthetic sequence
GYTFTSYAMN

SEQ ID NO: 66 - protein, 17 aa, synthetic construct
  REGION 1..17: note = Synthetic sequence
TINRYGGSTYYAASVKG

SEQ ID NO: 67 - protein, 17 aa, synthetic construct
  REGION 1..17: note = Synthetic sequence
TISRSGGSTYYAASVKG

SEQ ID NO: 68 - protein, 17 aa, synthetic construct
  REGION 1..17: note = Synthetic sequence
TINRYGGSTYYPDSFKG

SEQ ID NO: 69 - protein, 17 aa, synthetic construct
  REGION 1..17: note = Synthetic sequence
TINRYGGSTYYAQKFQG

SEQ ID NO: 70 - protein, 17 aa, synthetic construct
  REGION 1..17: note = Synthetic sequence
IINRNGGSTYYAQKFQG

SEQ ID NO: 71 - protein, 17 aa, synthetic construct
  REGION 1..17: note = Synthetic sequence
TINRYGGSPYYAQGFTG

SEQ ID NO: 72 - protein, 17 aa, synthetic construct
  REGION 1..17: note = Synthetic sequence
TINRYGGNPYYAQGFTG

SEQ ID NO: 73 - protein, 10 aa, synthetic construct
  REGION 1..10: note = Synthetic sequence
  VARIANT 2: note = Xaa is selected among I or L
LXYYGNEGES

SEQ ID NO: 74 - protein, 10 aa, synthetic construct
  REGION 1..10: note = Synthetic sequence
  VARIANT 2: note = Xaa is selected among I or L
LXYYGNEGDT

SEQ ID NO: 75 - protein, 10 aa, synthetic construct
  REGION 1..10: note = Synthetic sequence
  VARIANT 2: note = Xaa is selected among I or L
LXYYGNEGET

SEQ ID NO: 76 - protein, 10 aa, synthetic construct
  REGION 1..10: note = Synthetic sequence
RASQSVSFMH

SEQ ID NO: 77 - protein, 10 aa, synthetic construct
  REGION 1..10: note = Synthetic sequence
RASQSVSFLH

SEQ ID NO: 78 - protein, 10 aa, synthetic construct
  REGION 1..10: note = Synthetic sequence
RASQGISFLA

SEQ ID NO: 79 - protein, 10 aa, synthetic construct
  REGION 1..10: note = Synthetic sequence
RASQSVSFLA

SEQ ID NO: 80 - protein, 10 aa, synthetic construct
  REGION 1..10: note = Synthetic sequence
RASQSISFLH

SEQ ID NO: 81 - protein, 7 aa, synthetic construct
  REGION 1..7: note = Synthetic sequence
DATKLTS

SEQ ID NO: 82 - protein, 7 aa, synthetic construct
  REGION 1..7: note = Synthetic sequence
DASKLTS

SEQ ID NO: 83 - protein, 7 aa, synthetic construct
  REGION 1..7: note = Synthetic sequence
DASKLES

SEQ ID NO: 84 - protein, 7 aa, synthetic construct
  REGION 1..7: note = Synthetic sequence
DATKSTS

SEQ ID NO: 85 - protein, 7 aa, synthetic construct
  REGION 1..7: note = Synthetic sequence
DASKSFS

SEQ ID NO: 86 - protein, 7 aa, synthetic construct
  REGION 1..7: note = Synthetic sequence
DATKRTT

SEQ ID NO: 87 - protein, 7 aa, synthetic construct
  REGION 1..7: note = Synthetic sequence
DASKSTS

SEQ ID NO: 88 - protein, 7 aa, synthetic construct
  REGION 1..7: note = Synthetic sequence
DASKRTT

SEQ ID NO: 89 - protein, 10 aa, synthetic construct
  REGION 1..10: note = Synthetic sequence
QQWQSKPPLT

SEQ ID NO: 90 - protein, 25 aa, synthetic construct
  REGION 1..25: note = Synthetic sequence
EVQLVASGGGLVQPGGSLKLSCAAS

SEQ ID NO: 91 - protein, 25 aa, synthetic construct [sequence omitted]

SEQ ID NO: 92 - protein, 25 aa, synthetic construct [sequence omitted]

SEQ ID NO: 93 - protein, 25 aa, synthetic construct
  REGION 1..25: note = Synthetic sequence
QVQLVQSGSELKKPGASVKVSCKAS

SEQ ID NO: 94 - protein, 14 aa, synthetic construct
  REGION 1..14: note = Synthetic sequence
WVRQTPDRRLELVA

SEQ ID NO: 95 - protein, 14 aa, synthetic construct
  REGION 1..14: note = Synthetic sequence
WVRQAPGKGLELVA

SEQ ID NO: 96 - protein, 14 aa, synthetic construct
  REGION 1..14: note = Synthetic sequence
WVRQAPGQGLELVA

SEQ ID NO: 97 - protein, 14 aa, synthetic construct
  REGION 1..14: note = Synthetic sequence
WVRQAPGQGLELVA

SEQ ID NO: 98 - protein, 14 aa, synthetic construct
  REGION 1..14: note = Synthetic sequence
WVRQAPGKGLELVS

SEQ ID NO: 99 - protein, 14 aa, synthetic construct
  REGION 1..14: note = Synthetic sequence
WVRQAPGQGLELVG

SEQ ID NO: 100 - protein, 14 aa, synthetic construct
  REGION 1..14: note = Synthetic sequence
WVRQAPGQGLELMG

SEQ ID NO: 101 - protein, 32 aa, synthetic construct
  REGION 1..32: note = Synthetic sequence
RFTISRDNAKNTLYLQMSSLKSEDTAMYYCPR

SEQ ID NO: 102 - protein, 32 aa, synthetic construct
  REGION 1..32: note = Synthetic sequence
RFTISRDNSKNTLYLQMNSLRAEDTAVYYCPK

SEQ ID NO: 103 - protein, 32 aa, synthetic construct
  REGION 1..32: note = Synthetic sequence
RVTITRDNSTSTLYMELSSLRSEDTAVYYCPR

SEQ ID NO: 104 - protein, 32 aa, synthetic construct
  REGION 1..32: note = Synthetic sequence
RFVISRDNSVSTLYLQISSLKAEDTAVYYCPR

SEQ ID NO: 105 - protein, 32 aa, synthetic construct
  REGION 1..32: note = Synthetic sequence
RVTITRDTSTSTVYMELSSLRSEDTAVYYCPR

SEQ ID NO: 106 - protein, 32 aa, synthetic construct
  REGION 1..32: note = Synthetic sequence
RFVISRDTSVSTAYLQISSLKAEDTAVYYCPR

SEQ ID NO: 107 - protein, 11 aa, synthetic construct
  REGION 1..11: note = Synthetic sequence
WGQGTTLTVSS

SEQ ID NO: 108 - protein, 11 aa, synthetic construct
  REGION 1..11: note = Synthetic sequence
WGQGTLVTVSS

SEQ ID NO: 109 - protein, 23 aa, synthetic construct
  REGION 1..23: note = Synthetic sequence
QIVLTQSPAIMSASPGEKVTMTC

SEQ ID NO: 110 - protein, 23 aa, synthetic construct
  REGION 1..23: note = Synthetic sequence
AIQLTQSPSSLSASVGDRVTITC

SEQ ID NO: 111 - protein, 23 aa, synthetic construct
  REGION 1..23: note = Synthetic sequence
EIVLTQSPDFQSVTPKEKVTITC

SEQ ID NO: 112 - protein, 23 aa, synthetic construct
  REGION 1..23: note = Synthetic sequence
EIVLTQSPATLSLSPGERATLSC

SEQ ID NO: 113 - protein, 15 aa, synthetic construct
  REGION 1..15: note = Synthetic sequence
WYQQKSGTSPKRWIY

SEQ ID NO: 114 - protein, 15 aa, synthetic construct
  REGION 1..15: note = Synthetic sequence
WYQQKPGKAPKRWIY

SEQ ID NO: 115 - protein, 15 aa, synthetic construct
  REGION 1..15: note = Synthetic sequence
WYQQKPDQSPKRWIY

SEQ ID NO: 116 - protein, 15 aa, synthetic construct
  REGION 1..15: note = Synthetic sequence
WYQQKPGQAPRRWIY

SEQ ID NO: 117 - protein, 15 aa, synthetic construct
  REGION 1..15: note = Synthetic sequence
WYQQKPGKAPKRLIY

SEQ ID NO: 118 - protein, 32 aa, synthetic construct
  REGION 1..32: note = Synthetic sequence
GVPARFSGSGSGTFYSLTISSMEAEDAATYYC

SEQ ID NO: 119 - protein, 32 aa, synthetic construct
  REGION 1..32: note = Synthetic sequence
GVPSRFSGSGSGTDYTLTISSLQPEDFATYYC

SEQ ID NO: 120 - protein, 32 aa, synthetic construct
  REGION 1..32: note = Synthetic sequence
GVPSRFSGSGSGTDYTLTINSLEAEDAATYYC

SEQ ID NO: 121 - protein, 32 aa, synthetic construct
  REGION 1..32: note = Synthetic sequence
GIPARFSGSGSGTDYTLTISSLEPEDFAVYYC

SEQ ID NO: 122 - protein, 32 aa, synthetic construct
  REGION 1..32: note = Synthetic sequence
GVPSRFSGSGSGTDFTLTISSLQPEDFATYYC

SEQ ID NO: 123 - protein, 10 aa, synthetic construct
  REGION 1..10: note = Synthetic sequence
FGPGTKLELK

SEQ ID NO: 124 - protein, 10 aa, synthetic construct
  REGION 1..10: note = Synthetic sequence
FGGGTKVEIK

SEQ ID NO: 125 - protein, 14 aa, synthetic construct
  REGION 1..14: note = Synthetic sequence
  VARIANT 4: note = Xaa is selected among Q or A
  VARIANT 7: note = Xaa is selected among D or G
  VARIANT 8: note = Xaa is selected among R or K
  VARIANT 9: note = Xaa is selected among R, G or Q
WVRXTPXXXLELVA

SEQ ID NO: 126 - protein, 32 aa, synthetic construct
  REGION 1..32: note = Synthetic sequence
  VARIANT 2: note = Xaa is selected among F or V
  VARIANT 3: note = Xaa is selected among T or V
  VARIANT 5: note = Xaa is selected among S or T
  VARIANT 9: note = Xaa is selected among A or S
  VARIANT 10: note = Xaa is selected among K, T or V
  VARIANT 11: note = Xaa is selected among N or S
  VARIANT 15: note = Xaa is selected among L or M
  VARIANT 16: note = Xaa is selected among Q or E
  VARIANT 17: note = Xaa is selected among M, L or I
  VARIANT 21: note = Xaa is selected among K or R
  VARIANT 22: note = Xaa is selected among S or A
  VARIANT 27: note = Xaa is selected among M or V
RXXIXRDNXXXTLYXXXSSLXXEDTAXYYCPR

SEQ ID NO: 127 - protein, 11 aa, synthetic construct
  REGION 1..11: note = Synthetic sequence
  VARIANT 6: note = Xaa is selected among T or L
  VARIANT 7: note = Xaa is selected among L or V
WGQGTXXTVSS

SEQ ID NO: 128 - protein, 23 aa, synthetic construct
  REGION 1..23: note = Synthetic sequence
  VARIANT 1: note = Xaa is selected among Q, A or E
  VARIANT 3: note = Xaa is selected among V or Q
  VARIANT 9: note = Xaa is selected among A, S or D
  VARIANT 10: note = Xaa is selected among I, S, F or T
  VARIANT 11: note = Xaa is selected among M, L or Q
  VARIANT 13: note = Xaa is selected among A, S or L
  VARIANT 14: note = Xaa is selected among S or V
  VARIANT 15: note = Xaa is selected among P, V or T
  VARIANT 16: note = Xaa is selected among G or P
  VARIANT 17: note = Xaa is selected among E, D or K
  VARIANT 18: note = Xaa is selected among K or R
  VARIANT 19: note = Xaa is selected among V or A
  VARIANT 21: note = Xaa is selected among M, I or L
XIXLTQSPXXXSXXXXXXXTXTC

SEQ ID NO: 129 - protein, 15 aa, synthetic construct
  REGION 1..15: note = Synthetic sequence
  VARIANT 6: note = Xaa is selected among S or P
  VARIANT 7: note = Xaa is selected among G or D
  VARIANT 8: note = Xaa is selected among T or K
  VARIANT 9: note = Xaa is selected among S or A
  VARIANT 11: note = Xaa is selected among K or R
WYQQKXXXXPXRWIY

SEQ ID NO: 130 - protein, 32 aa, synthetic construct
  REGION 1..32: note = Synthetic sequence
  VARIANT 2: note = Xaa is selected among V or I
  VARIANT 4: note = Xaa is selected among A or S
  VARIANT 14: note = Xaa is selected among F or D
  VARIANT 16: note = Xaa is selected among S or T
  VARIANT 20: note = Xaa is selected among S or N
  VARIANT 22: note = Xaa is selected among M or L
  VARIANT 23: note = Xaa is selected among E or Q
  VARIANT 24: note = Xaa is selected among A or P
  VARIANT 27: note = Xaa is selected among A or F
  VARIANT 29: note = Xaa is selected among T or V
GXPXRFSGSGSGTXYXLTIXSXXXEDXAXYYC

SEQ ID NO: 131 - protein, 11 aa, synthetic construct
  REGION 1..11: note = Synthetic sequence
  VARIANT 3: note = Xaa is selected among P or G
  VARIANT 7: note = Xaa is selected among L or V
  VARIANT 9: note = Xaa is selected among L or I
FGXGTKXEXKR

SEQ ID NO: 132 - protein, 32 aa, synthetic construct
  REGION 1..32: note = Synthetic sequence
GVPSRFSGSGSGTDFTLTINSLEAEDAATYYC

SEQ ID NO: 133 - DNA, 993 bp, synthetic construct
  misc_feature 1..993: note = Synthetic sequence
  source 1..993: mol_type = other DNA
gctagcaccaagggcccatcggtcttccccctggcaccctcctccaagagcacctctgggggcacagcggccctgggctgcctggtcaaggactacttccccgaaccggtgacggtgtcgtggaactcaggcgccctgaccagcggcgtgcacaccttcccggctgtcctacagtcctcaggactctactccctcagcagcgtggtgaccgtgccctccagcagcttgggcacccagacctacatctgcaacgtgaatcacaagcccagcaacaccaaggtggacaagaaagttgagcccaaatcttgtgacaaaactcacacatgcccaccgtgcccagcacctgaactcctggggggaccgtcagtcttcctcttccccccaaaacccaaggacaccctcatgatctcccggacccctgaggtcacatgcgtggtggtggacgtgagccacgaagaccctgaggtcaagttcaactggtacgtggacggcgtggaggtgcataatgccaagacaaagccgcgggaggagcagtacaacagcacgtaccgtgtggtcagcgtcctcaccgtcctgcaccaggactggctgaatggcaaggagtacaagtgcaaggtctccaacaaagccctcccagcccccatcgcgaaaaccatctccaaagccaaagggcagccccgagaaccacaggtgtacaccctgcccccatcccgggaggagatgaccaagaaccaggtcagcctgacctgcctggtcaaaggcttctatcccagcgacatcgccgtggagtgggagagcaatgggcagccggagaacaactacaagaccacgcctcccgtgctggactccgacggctccttcttcctctacagcaagctcaccgtggacaagagcaggtggcagcaggggaacgtcttctcatgctccgtgatgcatgaggctctgcacaaccactacacgcagaagagcctctccctgtctccgggtaaatga

SEQ ID NO: 134 - protein, 330 aa, synthetic construct
  REGION 1..330: note = Synthetic sequence
ASTKGPSVFPLAPSSKSTSGGTAALGCLVKDYFPEPVTVSWNSGALTSGVHTFPAVLQSSGLYSLSSVVTVPSSSLGTQTYICNVNHKPSNTKVDKKVEPKSCDKTHTCPPCPAPELLGGPSVFLFPPKPKDTLMISRTPEVTCVVVDVSHEDPEVKFNWYVDGVEVHNAKTKPREEQYNSTYRVVSVLTVLHQDWLNGKEYKCKVSNKALPAPIAKTISKAKGQPREPQVYTLPPSREEMTKNQVSLTCLVKGFYPSDIAVEWESNGQPENNYKTTPPVLDSDGSFFLYSKLTVDKSRWQQGNVFSCSVMHEALHNHYTQKSLSLSPGK

SEQ ID NO: 135 - DNA, 984 bp, synthetic construct
  misc_feature 1..984: note = Synthetic sequence
  source 1..984: mol_type = other DNA
gctagcaccaagggcccatcggtcttccccctggcgccctgctccaggagcacctccgagagcacagccgccctgggctgcctggtcaaggactacttccccgaaccggtgacggtgtcgtggaactcaggcgccctgaccagcggcgtgcacaccttcccggctgtcctacagtcctcaggactctactccctcagcagcgtggtgaccgtgccctccagcagcttgggcacgaagacctacacctgcaacgtagatcacaagcccagcaacaccaaggtggacaagagagttgagtccaaatatggtcccccatgcccaccatgcccagcacctgagttcctggggggaccatcagtcttcctgttccccccaaaacccaaggacactctcatgatctcccggacccctgaggtcacgtgcgtggtggtggacgtgagccaggaagaccccgaggtccagttcaactggtacgtggatggcgtggaggtgcataatgccaagacaaagccgcgggaggagcagttcaacagcacgtaccgtgtggtcagcgtcctcaccgtcctgcaccaggactggctgaacggcaaggagtacaagtgcaaggtctccaacaaaggcctcccgtcctccatcgagaaaaccatctccaaagccaaagggcagccccgagagccacaggtgtacaccctgcccccatcccaggaggagatgaccaagaaccaggtcagcctgacctgcctggtcaaaggcttctaccccagcgacatcgccgtggagtgggagagcaatgggcagccggagaacaactacaagaccacgcctcccgtgctggactccgacggctccttcttcctctacagcaggctaaccgtggacaagagcaggtggcaggaggggaatgtcttctcatgctccgtgatgcatgaggctctgcacaaccactacacacagaagagcctctccctgtctccgggtaaatga

SEQ ID NO: 136 - protein, 327 aa, synthetic construct
  REGION 1..327: note = Synthetic sequence
ASTKGPSVFPLAPCSRSTSESTAALGCLVKDYFPEPVTVSWNSGALTSGVHTFPAVLQSSGLYSLSSVVTVPSSSLGTKTYTCNVDHKPSNTKVDKRVESKYGPPCPPCPAPEFLGGPSVFLFPPKPKDTLMISRTPEVTCVVVDVSQEDPEVQFNWYVDGVEVHNAKTKPREEQFNSTYRVVSVLTVLHQDWLNGKEYKCKVSNKGLPSSIEKTISKAKGQPREPQVYTLPPSQEEMTKNQVSLTCLVKGFYPSDIAVEWESNGQPENNYKTTPPVLDSDGSFFLYSRLTVDKSRWQEGNVFSCSVMHEALHNHYTQKSLSLSPGK

SEQ ID NO: 137 - DNA, 321 bp, synthetic construct
  misc_feature 1..321: note = Synthetic sequence
  source 1..321: mol_type = other DNA
acggtggctgcaccatctgtcttcatcttcccgccatctgatgagcagttgaaatctggaactgcctctgttgtgtgcctgctgaataacttctatcccagagaggccaaagtacagtggaaggtggataacgccctccaatcgggtaactcccaggagagtgtcacagagcaggacagcaaggacagcacctacagcctcagcagcaccctgacgctgagcaaagcagactacgagaaacacaaagtctacgcctgcgaagtcacccatcagggcctgagctcgcccgtcacaaagagcttcaacaggggagagtgttag

SEQ ID NO: 138 - protein, 106 aa, synthetic construct
  REGION 1..106: note = Synthetic sequence
TVAAPSVFIFPPSDEQLKSGTASVVCLLNNFYPREAKVQWKVDNALQSGNSQESVTEQDSKDSTYSLSSTLTLSKADYEKHKVYACEVTHQGLSSPVTKSFNRGEC

SEQ ID NO: 139 - protein, 330 aa, synthetic construct [sequence omitted]

SEQ ID NO: 140 - protein, 326 aa, synthetic construct
  REGION 1..326: note = Synthetic sequence
ASTKGPSVFPLAPCSRSTSESTAALGCLVKDYFPEPVTVSWNSGALTSGVHTFPAVLQSSGLYSLSSVVTVPSSNFGTQTYTCNVDHKPSNTKVDKTVERKCCVECPPCPAPPVAGPSVFLFPPKPKDTLMISRTPEVTCVVVDVSHEDPEVQFNWYVDGVEVHNAKTKPREEQFNSTFRVVSVLTVVHQDWLNGKEYKCKVSNKGLPAPIEKTISKTKGQPREPQVYTLPPSREEMTKNQVSLTCLVKGFYPSDISVEWESNGQPENNYKTTPPMLDSDGSFFLYSKLTVDKSRWQQGNVFSCSVMHEALHNHYTQKSLSLSPGK

SEQ ID NO: 141 - protein, 327 aa, synthetic construct
  REGION 1..327: note = Synthetic sequence
ASTKGPSVFPLAPCSRSTSESTAALGCLVKDYFPEPVTVSWNSGALTSGVHTFPAVLQSSGLYSLSSVVTVPSSSLGTKTYTCNVDHKPSNTKVDKRVESKYGPPCPSCPAPEFLGGPSVFLFPPKPKDTLMISRTPEVTCVVVDVSQEDPEVQFNWYVDGVEVHNAKTKPREEQFNSTYRVVSVLTVLHQDWLNGKEYKCKVSNKGLPSSIEKTISKAKGQPREPQVYTLPPSQEEMTKNQVSLTCLVKGFYPSDIAVEWESNGQPENNYKTTPPVLDSDGSFFLYSRLTVDKSRWQEGNVFSCSVMHEALHNHYTQKSLSLSLGK

SEQ ID NO: 142 - protein, 214 aa, synthetic construct
  REGION 1..214: note = Synthetic sequence
QIVLTQSPAIMSASPGEKVTMTCSASSSVSFMHWYQQKSGTSPKRWIYDTTKLTSGVPARFSGSGSGTFYSLTISSMEAEDAATYYCQQWNSKPPLTFGPGTKLELKRTVAAPSVFIFPPSDEQLKSGTASVVCLLNNFYPREAKVQWKVDNALQSGNSQESVTEQDSKDSTYSLSSTLTLSKADYEKHKVYACEVTHQGLSSPVTKSFNRGEC

SEQ ID NO: 143 - protein, 449 aa, synthetic construct
  REGION 1..449: note = Synthetic sequence
EVQLVASGGGLVQPGGSLKLSCAASGFTFSSYGMSWVRQTPDRRLELVATINRYGGSTYYPDSVKGRFTISRDNAKNTLYLQMSSLKSEDTAMYYCPRLIYYGNEGDSWGQGTTLTVSSASTKGPSVFPLAPSSKSTSGGTAALGCLVKDYFPEPVTVSWNSGALTSGVHTFPAVLQSSGLYSLSSVVTVPSSSLGTQTYICNVNHKPSNTKVDKKVEPKSCDKTHTCPPCPAPELLGGPSVFLFPPKPKDTLMISRTPEVTCVVVDVSHEDPEVKFNWYVDGVEVHNAKTKPREEQYNSTYRVVSVLTVLHQDWLNGKEYKCKVSNKALPAPIEKTISKAKGQPREPQVYTLPPSRDELTKNQVSLTCLVKGFYPSDIAVEWESNGQPENNYKTTPPVLDSDGSFFLYSKLTVDKSRWQQGNVFSCSVMHEALHNHYTQKSLSLSPGK

SEQ ID NO: 144 - protein, 10 aa, synthetic construct
  REGION 1..10: note = Synthetic sequence
LIYYGNEGDS

SEQ ID NO: 145 - protein, 10 aa, synthetic construct
  REGION 1..10: note = Synthetic sequence
LIYYGNEGES

SEQ ID NO: 146 - protein, 10 aa, synthetic construct
  REGION 1..10: note = Synthetic sequence
LIYYGNEGDT

SEQ ID NO: 147 - protein, 10 aa, synthetic construct
  REGION 1..10: note = Synthetic sequence
LIYYGNEGET

SEQ ID NO: 148 - protein, 10 aa, synthetic construct
  REGION 1..10: note = Synthetic sequence
LLYYGNEGDS

SEQ ID NO: 149 - protein, 10 aa, synthetic construct
  REGION 1..10: note = Synthetic sequence
LLYYGNEGES

SEQ ID NO: 150 - protein, 10 aa, synthetic construct
  REGION 1..10: note = Synthetic sequence
LLYYGNEGDT

SEQ ID NO: 151 - protein, 10 aa, synthetic construct
  REGION 1..10: note = Synthetic sequence
LLYYGNEGET

SEQ ID NO: 152 - protein, 5 aa, synthetic construct
  REGION 1..5: note = Synthetic sequence
AMPGS